European Patent Application EP 4 321 624 A1, published February 14, 2024. Title: NOVEL SCREENING SYSTEM FOR DRUG TARGET ANTAGONIST BASED ON CELL LIFE/DEATH PHENOTYPE. Applicant: CENTER FOR EXCELLENCE IN MOLECULAR CELL SCIENCE, CHINESE ACADEMY OF SCIENCES. The sequence listing filed with the application follows.

SEQUENCE LISTING (2 sequences)

SEQ ID NO: 1 - protein, 395 aa, Artificial Sequence
  Amino acid sequence of FKBP12(F36V)-Caspase9
MGVQVETISPGDGRTFPKRGQTCVVHYTGMLEDGKKVDSSRDRNKPFKFMLGKQEVIRGWEEGVAQMSVGQRAKLTISPDYAYGATGHPGIIPPHATLVFDVELLKLESGGGSGFGDVGALESLRGNADLAYILSMEPCGHCLIINNVNFCRESGLRTRTGSNIDCEKLRRRFSSLHFMVEVKGDLTAKKMVLALLELAQQDHGALDCCVVVILSHGCQASHLQFPGAVYGTDGCPVSVEKIVNIFNGTSCPSLGGKPKLFFIQACGGEQKDHGFEVASTSPEDESPGSNPEPDATPFQEGLRTFDQLDAISSLPTPSDIFVSYSTFPGFVSWRDPKSGSWYVETLDDIFEQWAHSEDLQSLLLRVANAVSVKGIYKQMPGCFNFLRKKLFFKTS

SEQ ID NO: 2 - protein, 288 aa, Artificial Sequence
  Amino acid sequence of target protein PD1
MQIPQAPWPVVWAVLQLGWRPGWFLDSPDRPWNPPTFSPALLVVTEGDNATFTCSFSNTSESFVLNWYRMSPSNQTDKLAAFPEDRSQPGQDCRFRVTQLPNGRDFHMSVVRARRNDSGTYLCGAISLAPKAQIKESLRAELRVTERRAEVPTAHPSPSPRPAGQFQTLVVGVVGGLLGSLVLLVWVLAVICSRAARGTIGARRTGQPLKEDPSAVPVFSVDYGELDFQWREKTPEPPVPCVPEQTEYATIVFPSGMGTSSPARRGSADGPRSAQPLRPEDGHCSWPL